European Patent Application EP 4 190 811 A1, published June 7, 2023. Title: SPECIFIC HUMANIZED ANTIBODY  FOR ANTHRAX PROTECTIVE ANTIGEN AND METHOD FOR MANUFACTURING THEROF. Applicant: AGENCY FOR DEFENSE DEVELOPMENT. The sequence listing filed with the application follows.

SEQUENCE LISTING (16 sequences)

SEQ ID NO: 1 - protein, 233 aa, Artificial Sequence
  Light Chain of antibody for anthrax protective antigen
  SIGNAL (1)..(19)
  SITE (46)..(51): CDR1
  SITE (69)..(71): CDR2
  SITE (108)..(116): CDR3
MYLGLNYVFIVFLLNGVQSDIQMTQSPSSLSASVGDRVTITCRASQGISSWLAWYQQKPGKAPKLLIYKASSLQSGVPSRFSGSRSGTDFTLTISSLQPEDFATYYCQHSYGTPYSFGQGTKVEIKRTVAAPSVFIFPPSDEQLKSGTASVVCLLNNFYPREAKVQWKVDNALQSGNSQESVTEQDSKDSTYSLSSTLTLSKADYEKHKVYACEVTHQGLSSPVTKSFNRGEC

SEQ ID NO: 2 - protein, 468 aa, Artificial Sequence
  Heavy Chain of antibody for anthrax protective antigen
  SIGNAL (1)..(19)
  SITE (45)..(52): CDR1
  SITE (70)..(77): CDR2
  SITE (116)..(127): CDR3
MYLGLNYVFIVFLLNGVQSEVQLVESGGGLVQPGGSLRLSCAVSGGSISGYWWGWIRQAPGKGLEWIGCIGGSSGTTYYNPSLKSRVTISADTSKNTAYLQMNSLRAEDTAVYYCARGGFSCSYYSNWGQGTLVTVSSASTKGPSVFPLAPSSKSTSGGTAALGCLVKDYFPEPVTVSWNSGALTSGVHTFPAVLQSSGLYSLSSVVTVPSSSLGTQTYICNVNHKPSNTKVDKKVEPKSCDKTHTCPPCPAPELLGGPSVFLFPPKPKDTLMISRTPEVTCVVVDVSHEDPEVKFNWYVDGVEVHNAKTKPREEQYNSTYRVVSVLTVLHQDWLNGKEYKCKVSNKALPAPIEKTISKAKGQPREPQVYTLPPSRDELTKNQVSLTCLVKGFYPSDIAVEWESNGQPENNYKTTPPVLDSDGSFFLYSKLTVDKSRWQQGNVFSCSVMHEALHNHYTQKSLSLSPGK

SEQ ID NO: 3 - DNA, 702 bp, Artificial Sequence
  Light Chain of antibody for anthrax protective antigen
  misc_feature (136)..(153): CDR1
  misc_feature (205)..(213): CDR2
  misc_feature (322)..(348): CDR3
atgtacctgggcctgaactacgtgttcatcgtgtttctgctgaacggcgtgcagtccgacatccagatgacccagtccccctcctccctgtccgcctccgtgggcgacagagtgaccatcacctgtcgggcctcccagggcatctcctcctggctggcctggtatcagcagaagcccggcaaggcccccaagctgctgatctacaaggcctcctccctgcagtccggcgtgccctccagattctccggctccagatccggcaccgacttcaccctgaccatctcctccctgcagcccgaggacttcgccacctactactgccagcactcctacggcaccccctactccttcggccagggcaccaaggtggaaatcaagcgtacggtggccgctccctccgtgttcatcttcccaccctccgacgagcagctgaagtccggcaccgcctccgtcgtgtgcctgctgaacaacttctacccccgcgaggccaaggtgcagtggaaggtggacaacgccctgcagtccggcaactcccaggaatccgtcaccgagcaggactccaaggactctacctactccctgtcctccaccctgaccctgtccaaggccgactacgagaagcacaaggtgtacgcctgcgaagtgacccaccagggcctgtcctccccagtgaccaagtccttcaaccggggcgagtgttga

SEQ ID NO: 4 - DNA, 1407 bp, Artificial Sequence
  Heavy Chain of antibody for anthrax protective antigen
  misc_feature (133)..(156): CDR1
  misc_feature (208)..(231): CDR2
  misc_feature (346)..(381): CDR3
atgtacctgggcctgaactacgtgttcatcgtgtttctgctgaacggcgtgcagtccgaggtgcagctggtggaatctggcggcggactggtgcagcctggcggctccctgagactgtcttgtgccgtgtccggcggctccatctccggctattggtggggctggattcggcaggctcccggcaagggcctggaatggatcggctgcatcggcggctcctccggcaccacctactacaacccctccctgaagtccagagtgaccatctccgccgacacctccaagaacaccgcctacctgcagatgaactccctgcgggccgaggacaccgccgtgtactactgtgccagaggcggcttctcctgctcctactactccaactggggccagggcaccctggtcaccgtgtcctccgcctccaccaagggcccctccgtgttccctctggccccatcctccaagtccacctctggcggcaccgccgctctgggctgcctggtcaaggactacttccccgaaccggtgacagtgtcctggaactctggcgccctgacctccggcgtgcacaccttccctgccgtgctgcagtcctccggcctgtactccctgtcctccgtcgtgaccgtgccctcatcctccctgggcacccagacctacatctgcaacgtgaaccacaagccctccaacaccaaggtggacaagaaggtggaacccaagtcctgcgacaagacccacacctgtcccccctgccctgcccctgaactgctgggcggaccttccgtgttcctgttccccccaaagcccaaggacaccctgatgatctcccggacccccgaagtgacctgcgtggtggtggacgtgtcccacgaggaccctgaagtgaagtttaattggtacgtggacggcgtggaagtgcacaacgccaagaccaagcccagagaggaacagtacaactccacctaccgggtggtgtccgtgctgacagtgctgcaccaggactggctgaacggcaaagagtacaagtgcaaggtgtccaacaaggccctgcctgcccccatcgaaaagaccatctccaaggctaagggccagccccgcgagccccaggtgtacaccctgcctccatctcgggacgagctgaccaagaaccaggtgtccctgacatgtctggtcaagggcttctacccctccgatatcgccgtggaatgggagtccaacggccagcccgagaacaactacaagaccaccccccctgtgctggactccgacggctcattcttcctgtactccaagctgaccgtggacaagtcccggtggcagcagggcaacgtgttctcctgctccgtgatgcacgaggccctgcacaaccactacacccagaagtccctgtccctgtctcccggcaagtga

SEQ ID NO: 5 - protein, 6 aa, Artificial Sequence
  Light Chain CDR1
QGISSW

SEQ ID NO: 6 - protein, 3 aa, Artificial Sequence
  Light Chain CDR2
KAS

SEQ ID NO: 7 - protein, 9 aa, Artificial Sequence
  Light Chain CDR3
QHSYGTPYS

SEQ ID NO: 8 - protein, 8 aa, Artificial Sequence
  Heavy Chain CDR1
GGSISGYW

SEQ ID NO: 9 - protein, 8 aa, Artificial Sequence
  Heavy Chain CDR2
IGGSSGTT

SEQ ID NO: 10 - protein, 12 aa, Artificial Sequence
  Heavy Chain CDR3
ARGGFSCSYYSN

SEQ ID NO: 11 - DNA, 18 bp, Artificial Sequence
  Light Chain CDR1
cagggcatctcctcctgg

SEQ ID NO: 12 - DNA, 9 bp, Artificial Sequence
  Light Chain CDR2
aaggcctcc

SEQ ID NO: 13 - DNA, 27 bp, Artificial Sequence
  Light Chain CDR3
cagcactcctacggcaccccctactcc

SEQ ID NO: 14 - DNA, 24 bp, Artificial Sequence
  Heavy Chain CDR1
ggcggctccatctccggctattgg

SEQ ID NO: 15 - DNA, 24 bp, Artificial Sequence
  Heavy Chain CDR2
atcggcggctcctccggcaccacc

SEQ ID NO: 16 - DNA, 36 bp, Artificial Sequence
  Heavy Chain CDR3
gccagaggcggcttctcctgctcctactactccaac